European Patent Application EP 4 230 226 A1, published August 23, 2023. Title: Pharmaceutical composition for treating retinal or choroidal disease comprising an ACTA2 inhibitor as an active ingredient. Applicant: THE ASAN FOUNDATION University of Ulsan Foundation For Industry Cooperation. The sequence listing filed with the application follows.

SEQUENCE LISTING (9 sequences)

SEQ ID NO: 1 - protein, 377 aa, Artificial Sequence
  ACTA2, protein, NP_001135417.1
MCEEEDSTALVCDNGSGLCKAGFAGDDAPRAVFPSIVGRPRHQGVMVGMGQKDSYVGDEAQSKRGILTLKYPIEHGIITNWDDMEKIWHHSFYNELRVAPEEHPTLLTEAPLNPKANREKMTQIMFETFNVPAMYVAIQAVLSLYASGRTTGIVLDSGDGVTHNVPIYEGYALPHAIMRLDLAGRDLTDYLMKILTERGYSFVTTAEREIVRDIKEKLCYVALDFENEMATAASSSSLEKSYELPDGQVITIGNERFRCPETLFQPSFIGMESAGIHETTYNSIMKCDIDIRKDLYANNVLSGGTTMYPGIADRMQKEITALAPSTMKIKIIAPPERKYSVWIGGSILASLSTFQQMWISKQEYDEAGPSIVHRKCF

SEQ ID NO: 2 - DNA, 1805 bp, Artificial Sequence
  ACTA2, mRNA, NM_001141945.2
gcaggctctctccccgcccccgcggggcggcgcgcactcacccacccgcgccggagcggacctttggcttggcttgtcagggcttgtccaggagttccgctcctctctccaaccggggtccccctccagcgaccctaaagcttcccagacttccgcttcaattcctgtccgcaccccacgcccacctcaacgtggagcgcagtggtctccgaggagcgccggagctgccccgcctgcccagcggggtcagcacttcgcatcaaggcccaagaaaagcaagtcctccagcgttctgagcacccgggcctgagggaaggtcctaacagcccccgggagccagtctccaacgcctcccgcagcagcccgccgctcccaggtgcccgcgtgcgccgctgccgccgcaatcccgcacgcgtcccgcgcccgccccactttgcctatccccgggactaagacgggaatcctgtgaagcagctccagctatgtgtgaagaagaggacagcactgccttggtgtgtgacaatggctctgggctctgtaaggccggctttgctggggacgatgctcccagggctgttttcccatccattgtgggacgtcccagacatcagggggtgatggtgggaatgggacaaaaagacagctacgtgggtgacgaagcacagagcaaaagaggaatcctgaccctgaagtacccgatagaacatggcatcatcaccaactgggacgacatggaaaagatctggcaccactctttctacaatgagcttcgtgttgcccctgaagagcatcccaccctgctcacggaggcacccctgaaccccaaggccaaccgggagaaaatgactcaaattatgtttgagactttcaatgtcccagccatgtatgtggctatccaggcggtgctgtctctctatgcctctggacgcacaactggcatcgtgctggactctggagatggtgtcacccacaatgtccccatctatgagggctatgccttgccccatgccatcatgcgtctggatctggctggccgagatctcactgactacctcatgaagatcctgactgagcgtggctattccttcgttactactgctgagcgtgagattgtccgggacatcaaggagaaactgtgttatgtagctctggactttgaaaatgagatggccactgccgcatcctcatcctcccttgagaagagttacgagttgcctgatgggcaagtgatcaccatcggaaatgaacgtttccgctgcccagagaccctgttccagccatccttcatcgggatggagtctgctggcatccatgaaaccacctacaacagcatcatgaagtgtgatattgacatcaggaaggacctctatgctaacaatgtcctatcagggggcaccactatgtaccctggcattgccgaccgaatgcagaaggagatcacggccctagcacccagcaccatgaagatcaagatcattgcccctccggagcgcaaatactctgtctggatcggtggctccatcctggcctctctgtccaccttccagcagatgtggatcagcaaacaggaatacgatgaagccgggccttccattgtccaccgcaaatgcttctaaaacactttcctgctcctctctgtctctagcacacaactgtgaatgtcctgtggaattatgccttcagttcttttccaaatcattcctagccaaagctctgactcgttacctatgtgttttttaataaatctgaaataggctactggtaaaaaaaaaaaaaaaaaaaaaaaaaaaaaaaaaaaaaaaaaa

SEQ ID NO: 3 - RNA, 19 nt, Artificial Sequence
  siRNA 1_sense
cguacacaagacucucaca

SEQ ID NO: 4 - RNA, 19 nt, Artificial Sequence
  siRNA 1_antisense
ugugagagucuuguguacg

SEQ ID NO: 5 - RNA, 19 nt, Artificial Sequence
  siRNA 2_sense
cacuaugcaccuggaucau

SEQ ID NO: 6 - RNA, 19 nt, Artificial Sequence
  siRNA 2_antisense
augauccaggugcauagug

SEQ ID NO: 7 - RNA, 19 nt, Artificial Sequence
  siRNA 3_sense
gauuuguuacucgugguuu

SEQ ID NO: 8 - RNA, 19 nt, Artificial Sequence
  siRNA 3_antisense
aaaccacgaguaacaaauc

SEQ ID NO: 9 - RNA, 69 nt, Artificial Sequence
  has-miR-4524a-3p
gaacgauagcagcaugaaccugucucacugcagaauuauuuugagacaggcuuaugcugcuauccuuca